European Patent Specification EP 3 837 551 B1, published February 21, 2024. Title: Modulators of the function of Factor H-related protein 1 and uses thereof in the control of inflammation. Applicant: Leibniz-Institut für Naturstoff-Forschung und Infektionsbiologie - Hans Knöll Institut. The sequence listing filed with the application follows.

SEQUENCE LISTING (7 sequences)

SEQ ID NO: 1 - DNA, 66 bp, Homo sapiens
caagttcctacaggggaagttttctcttactactgtgagagaattttgtgtctccttcaaaatcct

SEQ ID NO: 2 - DNA, 20 bp, Homo sapiens
gctaagtcctgccctcattt

SEQ ID NO: 3 - DNA, 20 bp, Homo sapiens
gtacaggtctttgcggatgt

SEQ ID NO: 4 - DNA, 22 bp, Homo sapiens
ctctcacctctcctactcactt

SEQ ID NO: 5 - DNA, 20 bp, Homo sapiens
tcagaatgtgggagcgaatg

SEQ ID NO: 6 - DNA, 21 bp, Homo sapiens
ccagggacctctctctaatca

SEQ ID NO: 7 - DNA, 20 bp, Homo sapiens
tcagcttgagggtttgctac